European Patent Application EP 4 212 616 A1, published July 19, 2023. Title: Method for preparing stem cells having improved engraftment. Applicant: GENEROATH CO.,LTD. The sequence listing filed with the application follows.

SEQUENCE LISTING (2 sequences)

SEQ ID NO: 1 - DNA, 756 bp, Artificial Sequence
  AIMP2 variant of nucleic acid
atgccgatgtaccaggtaaagccctatcacgggggcggcgcgcctctccgtgtggagcttcccacctgcatgtaccggctccccaacgtgcacggcaggagctacggcccagcgccgggcgctggccacgtgcaggattacggggcgctgaaagacatcgtgatcaacgcaaacccggcctcccctcccctctccctgcttgtgctgcacaggctgctctgtgagcacttcagggtcctgtccacggtgcacacgcactcctcggtcaagagcgtgcctgaaaaccttctcaagtgctttggagaacagaataaaaaacagccccgccaagactatcagctgggattcactttaatttggaagaatgtgccgaagacgcagatgaaattcagcatccagacgatgtgccccatcgaaggcgaagggaacattgcacgtttcttgttctctctgtttggccagaagcataatgctgtcaacgcaacccttatagatagctgggtagatattgcgatttttcagttaaaagagggaagcagtaaagaaaaagccgctgttttccgctccatgaactctgctcttgggaagagcccttggctcgctgggaatgaactcaccgtagcagacgtggtgctgtggtctgtactccagcagatcggaggctgcagtgtgacagtgccagccaatgtgcagaggtggatgaggtcttgtgaaaacctggctccttttaacacggccctcaagctccttaagtga

SEQ ID NO: 2 - protein, 251 aa, Artificial Sequence
  AIMP2 variant of amino acid
MPMYQVKPYHGGGAPLRVELPTCMYRLPNVHGRSYGPAPGAGHVQDYGALKDIVINANPASPPLSLLVLHRLLCEHFRVLSTVHTHSSVKSVPENLLKCFGEQNKKQPRQDYQLGFTLIWKNVPKTQMKFSIQTMCPIEGEGNIARFLFSLFGQKHNAVNATLIDSWVDIAIFQLKEGSSKEKAAVFRSMNSALGKSPWLAGNELTVADVVLWSVLQQIGGCSVTVPANVQRWMRSCENLAPFNTALKLLK